European Patent Application EP 4 435 011 A1, published September 25, 2024. Title: 一种以白介素15为活性成份的融合蛋白构建体及其应用. Applicant: 中国科学院生物物理研究所. Application CN. The sequence listing filed with the application follows.

SEQUENCE LISTING (21 sequences)

SEQ ID NO: 1 - protein, 114 aa, Mus musculus
NWIDVRYDLEKIESLIQSIHIDTTLYTDSDFHPSCKVTAMNCFLLELQVILHEYSNMTLNETVRNVLYLANSTLSSNKNVAESGCKECEELEEKTFTEFLQSFIRIVQMFINTS

SEQ ID NO: 2 - protein, 224 aa, Homo sapiens
EPKSSDKTHTCPPCPAPELLGGPSVFLFPPKPKDTLMISRTPEVTCVVVDVSHEDPEVKFNWYVDGVEVHNAKTKPREEQYNSTYRVVSVLTVLHQDWLNGKEYKCKVSNKALPAPIEKTISKAKGQPREPQVYTLPPSRDELTKNQVSLTCLVKGFYPSDIAVEWESNGQPENNYKTTPPVLDSDGSFFLYSKLTVDKSRWQQGNVFSCSVMHEALHNHYTQK

SEQ ID NO: 3 - protein, 78 aa, Mus musculus
GTTCPPPVSIEHADIRVKNYSVNSRERYVCNSGFKRKAGTSTLIECVINKNTNVAHWTTPSLKCIRDPSLAHYSPVPT

SEQ ID NO: 4 - protein, 217 aa, Mus musculus
YELTQPPSASVNVGETVKITCSGDQLPKYFADWFHQRSDQTILQVIYDDNKRPSGIPERISGSSSGTTATLTIRDVRAEDEGDYYCFSGYVDSDSKLYVFGSGTQLTVLGRTVAAPSVFIFPPSDEQLKSGTASVVCLLNNFYPREAKVQWKVDNALQSGNSQESVTEQDSKDSTYSLSSTLTLSKADYEKHKVYACEVTHQGLSSPVTKSFNRGEC

SEQ ID NO: 5 - protein, 225 aa, Mus musculus
EVRLLESGGGLVKPEGSLKLSCVASGFTFSDYFMSWVRQAPGKGLEWVAHIYTKSYNYATYYSGSVKGRFTISRDDSRSMVYLQMNNLRTEDTATYYCTRDGSGYPSLDFWGQGTQVTVSSAASTKGPSVFPLAPSSKSTSGGTAALGCLVKDYFPEPVTVSWNSGALTSGVHTFPAVLQSSGLYSLSSVVTVPSSSLGTQTYICNVNHKPSNTKVDKRVEPKSC

SEQ ID NO: 6 - protein, 26 aa, synthetic construct
SGGGSGGGGSGGGGSGGGGSGGGSLQ

SEQ ID NO: 7 - protein, 471 aa, synthetic construct
KLATMETDTLLLWVLLLWVPGSTGEPKSSDKTHTCPPCPAPELLGGPSVFLFPPKPKDTLMISRTPEVTCVVVDVSHEDPEVKFNWYVDGVEVHNAKTKPREEQYNSTYRVVSVLTVLHQDWLNGKEYKCKVSNKALPAPIEKTISKAKGQPREPQVYTLPPSRDELTKNQVSLTCLVKGFYPSDIAVEWESNGQPENNYKTTPPVLDSDGSFFLYSKLTVDKSRWQQGNVFSCSVMHEALHNHYTQKGGGGSGTTCPPPVSIEHADIRVKNYSVNSRERYVCNSGFKRKAGTSTLIECVINKNTNVAHWTTPSLKCIRDPSLAHYSPVPTSGGGSGGGGSGGGGSGGGGSGGGSLQNWIDVRYDLEKIESLIQSIHIDTTLYTDSDFHPSCKVTAMNCFLLELQVILHEYSNMTLNETVRNVLYLANSTLSSNKNVAESGCKECEELEEKTFTEFLQSFIRIVQMFINTS

SEQ ID NO: 8 - protein, 471 aa, synthetic construct
KLATMETDTLLLWVLLLWVPGSTGEPKSSDKTHTCPPCPAPELLGGPSVFLFPPKPKDTLMISRTPEVTCVVVDVSHEDPEVKFNWYVDGVEVHNAKTKPREEQYNSTYRVVSVLTVLHQDWLNGKEYKCKVSNKALPAPIEKTISKAKGQPREPQVYTLPPSRDELTKNQVSLTCLVKGFYPSDIAVEWESNGQPENNYKTTPPVLDSDGSFFLYSKLTVDKSRWQQGNVFSCSVMHEALHNHYTQKGGGGSNWIDVRYDLEKIESLIQSIHIDTTLYTDSDFHPSCKVTAMNCFLLELQVILHEYSNMTLNETVRNVLYLANSTLSSNKNVAESGCKECEELEEKTFTEFLQSFIRIVQMFINTSSGGGSGGGGSGGGGSGGGGSGGGSLQGTTCPPPVSIEHADIRVKNYSVNSRERYVCNSGFKRKAGTSTLIECVINKNTNVAHWTTPSLKCIRDPSLAHYSPVPT

SEQ ID NO: 9 - protein, 915 aa, synthetic construct
YELTQPPSASVNVGETVKITCSGDQLPKYFADWFHQRSDQTILQVIYDDNKRPSGIPERISGSSSGTTATLTIRDVRAEDEGDYYCFSGYVDSDSKLYVFGSGTQLTVLGRTVAAPSVFIFPPSDEQLKSGTASVVCLLNNFYPREAKVQWKVDNALQSGNSQESVTEQDSKDSTYSLSSTLTLSKADYEKHKVYACEVTHQGLSSPVTKSFNRGECKLATMETDTLLLWVLLLWVPGSTGEVRLLESGGGLVKPEGSLKLSCVASGFTFSDYFMSWVRQAPGKGLEWVAHIYTKSYNYATYYSGSVKGRFTISRDDSRSMVYLQMNNLRTEDTATYYCTRDGSGYPSLDFWGQGTQVTVSSAASTKGPSVFPLAPSSKSTSGGTAALGCLVKDYFPEPVTVSWNSGALTSGVHTFPAVLQSSGLYSLSSVVTVPSSSLGTQTYICNVNHKPSNTKVDKRVEPKSCRTEPKSSDKTHTCPPCPAPELLGGPSVFLFPPKPKDTLMISRTPEVTCVVVDVSHEDPEVKFNWYVDGVEVHNAKTKPREEQYNSTYRVVSVLTVLHQDWLNGKEYKCKVSNKALPAPIEKTISKAKGQPREPQVYTLPPSRDELTKNQVSLTCLVKGFYPSDIAVEWESNGQPENNYKTTPPVLDSDGSFFLYSKLTVDKSRWQQGNVFSCSVMHEALHNHYTQKGGGGSGTTCPPPVSIEHADIRVKNYSVNSRERYVCNSGFKRKAGTSTLIECVINKNTNVAHWTTPSLKCIRDPSLAHYSPVPTSGGGSGGGGSGGGGSGGGGSGGGSLQNWIDVRYDLEKIESLIQSIHIDTTLYTDSDFHPSCKVTAMNCFLLELQVILHEYSNMTLNETVRNVLYLANSTLSSNKNVAESGCKECEELEEKTFTEFLQSFIRIVQMFINTS

SEQ ID NO: 10 - protein, 915 aa, synthetic construct
YELTQPPSASVNVGETVKITCSGDQLPKYFADWFHQRSDQTILQVIYDDNKRPSGIPERISGSSSGTTATLTIRDVRAEDEGDYYCFSGYVDSDSKLYVFGSGTQLTVLGRTVAAPSVFIFPPSDEQLKSGTASVVCLLNNFYPREAKVQWKVDNALQSGNSQESVTEQDSKDSTYSLSSTLTLSKADYEKHKVYACEVTHQGLSSPVTKSFNRGECKLATMETDTLLLWVLLLWVPGSTGEVRLLESGGGLVKPEGSLKLSCVASGFTFSDYFMSWVRQAPGKGLEWVAHIYTKSYNYATYYSGSVKGRFTISRDDSRSMVYLQMNNLRTEDTATYYCTRDGSGYPSLDFWGQGTQVTVSSAASTKGPSVFPLAPSSKSTSGGTAALGCLVKDYFPEPVTVSWNSGALTSGVHTFPAVLQSSGLYSLSSVVTVPSSSLGTQTYICNVNHKPSNTKVDKRVEPKSCRTEPKSSDKTHTCPPCPAPELLGGPSVFLFPPKPKDTLMISRTPEVTCVVVDVSHEDPEVKFNWYVDGVEVHNAKTKPREEQYNSTYRVVSVLTVLHQDWLNGKEYKCKVSNKALPAPIEKTISKAKGQPREPQVYTLPPSRDELTKNQVSLTCLVKGFYPSDIAVEWESNGQPENNYKTTPPVLDSDGSFFLYSKLTVDKSRWQQGNVFSCSVMHEALHNHYTQKGGGGSNWIDVRYDLEKIESLIQSIHIDTTLYTDSDFHPSCKVTAMNCFLLELQVILHEYSNMTLNETVRNVLYLANSTLSSNKNVAESGCKECEELEEKTFTEFLQSFIRIVQMFINTSSGGGSGGGGSGGGGSGGGGSGGGSLQGTTCPPPVSIEHADIRVKNYSVNSRERYVCNSGFKRKAGTSTLIECVINKNTNVAHWTTPSLKCIRDPSLAHYSPVPT

SEQ ID NO: 11 - protein, 481 aa, synthetic construct
KLATMETDTLLLWVLLLWVPGSTGEPKSSDKTHTCPPCPAPELLGGPSVFLFPPKPKDTLMISRTPEVTCVVVDVSHEDPEVKFNWYVDGVEVHNAKTKPREEQYNSTYRVVSVLTVLHQDWLNGKEYKCKVSNKALPAPIEKTISKAKGQPREPQVYTLPPSRDELTKNQVSLTCLVKGFYPSDIAVEWESNGQPENNYKTTPPVLDSDGSFFLYSKLTVDKSRWQQGNVFSCSVMHEALHNHYTQKGGGGSGGGGSGGGGSNWIDVRYDLEKIESLIQSIHIDTTLYTDSDFHPSCKVTAMNCFLLELQVILHEYSNMTLNETVRNVLYLANSTLSSNKNVAESGCKECEELEEKTFTEFLQSFIRIVQMFINTSSGGGSGGGGSGGGGSGGGGSGGGSLQGTTCPPPVSIEHADIRVKNYSVNSRERYVCNSGFKRKAGTSTLIECVINKNTNVAHWTTPSLKCIRDPSLAHYSPVPT

SEQ ID NO: 12 - protein, 925 aa, synthetic construct
YELTQPPSASVNVGETVKITCSGDQLPKYFADWFHQRSDQTILQVIYDDNKRPSGIPERISGSSSGTTATLTIRDVRAEDEGDYYCFSGYVDSDSKLYVFGSGTQLTVLGRTVAAPSVFIFPPSDEQLKSGTASVVCLLNNFYPREAKVQWKVDNALQSGNSQESVTEQDSKDSTYSLSSTLTLSKADYEKHKVYACEVTHQGLSSPVTKSFNRGECKLATMETDTLLLWVLLLWVPGSTGEVRLLESGGGLVKPEGSLKLSCVASGFTFSDYFMSWVRQAPGKGLEWVAHIYTKSYNYATYYSGSVKGRFTISRDDSRSMVYLQMNNLRTEDTATYYCTRDGSGYPSLDFWGQGTQVTVSSAASTKGPSVFPLAPSSKSTSGGTAALGCLVKDYFPEPVTVSWNSGALTSGVHTFPAVLQSSGLYSLSSVVTVPSSSLGTQTYICNVNHKPSNTKVDKRVEPKSCRTEPKSSDKTHTCPPCPAPELLGGPSVFLFPPKPKDTLMISRTPEVTCVVVDVSHEDPEVKFNWYVDGVEVHNAKTKPREEQYNSTYRVVSVLTVLHQDWLNGKEYKCKVSNKALPAPIEKTISKAKGQPREPQVYTLPPSRDELTKNQVSLTCLVKGFYPSDIAVEWESNGQPENNYKTTPPVLDSDGSFFLYSKLTVDKSRWQQGNVFSCSVMHEALHNHYTQKGGGGSGGGGSGGGGSNWIDVRYDLEKIESLIQSIHIDTTLYTDSDFHPSCKVTAMNCFLLELQVILHEYSNMTLNETVRNVLYLANSTLSSNKNVAESGCKECEELEEKTFTEFLQSFIRIVQMFINTSSGGGSGGGGSGGGGSGGGGSGGGSLQGTTCPPPVSIEHADIRVKNYSVNSRERYVCNSGFKRKAGTSTLIECVINKNTNVAHWTTPSLKCIRDPSLAHYSPVPT

SEQ ID NO: 13 - protein, 491 aa, synthetic construct
KLATMETDTLLLWVLLLWVPGSTGEPKSSDKTHTCPPCPAPELLGGPSVFLFPPKPKDTLMISRTPEVTCVVVDVSHEDPEVKFNWYVDGVEVHNAKTKPREEQYNSTYRVVSVLTVLHQDWLNGKEYKCKVSNKALPAPIEKTISKAKGQPREPQVYTLPPSRDELTKNQVSLTCLVKGFYPSDIAVEWESNGQPENNYKTTPPVLDSDGSFFLYSKLTVDKSRWQQGNVFSCSVMHEALHNHYTQKGGGGSGGGGSGGGGSGGGGSGGGGSNWIDVRYDLEKIESLIQSIHIDTTLYTDSDFHPSCKVTAMNCFLLELQVILHEYSNMTLNETVRNVLYLANSTLSSNKNVAESGCKECEELEEKTFTEFLQSFIRIVQMFINTSSGGGSGGGGSGGGGSGGGGSGGGSLQGTTCPPPVSIEHADIRVKNYSVNSRERYVCNSGFKRKAGTSTLIECVINKNTNVAHWTTPSLKCIRDPSLAHYSPVPT

SEQ ID NO: 14 - protein, 935 aa, synthetic construct
YELTQPPSASVNVGETVKITCSGDQLPKYFADWFHQRSDQTILQVIYDDNKRPSGIPERISGSSSGTTATLTIRDVRAEDEGDYYCFSGYVDSDSKLYVFGSGTQLTVLGRTVAAPSVFIFPPSDEQLKSGTASVVCLLNNFYPREAKVQWKVDNALQSGNSQESVTEQDSKDSTYSLSSTLTLSKADYEKHKVYACEVTHQGLSSPVTKSFNRGECKLATMETDTLLLWVLLLWVPGSTGEVRLLESGGGLVKPEGSLKLSCVASGFTFSDYFMSWVRQAPGKGLEWVAHIYTKSYNYATYYSGSVKGRFTISRDDSRSMVYLQMNNLRTEDTATYYCTRDGSGYPSLDFWGQGTQVTVSSAASTKGPSVFPLAPSSKSTSGGTAALGCLVKDYFPEPVTVSWNSGALTSGVHTFPAVLQSSGLYSLSSVVTVPSSSLGTQTYICNVNHKPSNTKVDKRVEPKSCRTEPKSSDKTHTCPPCPAPELLGGPSVFLFPPKPKDTLMISRTPEVTCVVVDVSHEDPEVKFNWYVDGVEVHNAKTKPREEQYNSTYRVVSVLTVLHQDWLNGKEYKCKVSNKALPAPIEKTISKAKGQPREPQVYTLPPSRDELTKNQVSLTCLVKGFYPSDIAVEWESNGQPENNYKTTPPVLDSDGSFFLYSKLTVDKSRWQQGNVFSCSVMHEALHNHYTQKGGGGSGGGGSGGGGSGGGGSGGGGSNWIDVRYDLEKIESLIQSIHIDTTLYTDSDFHPSCKVTAMNCFLLELQVILHEYSNMTLNETVRNVLYLANSTLSSNKNVAESGCKECEELEEKTFTEFLQSFIRIVQMFINTSSGGGSGGGGSGGGGSGGGGSGGGSLQGTTCPPPVSIEHADIRVKNYSVNSRERYVCNSGFKRKAGTSTLIECVINKNTNVAHWTTPSLKCIRDPSLAHYSPVPT

SEQ ID NO: 15 - protein, 114 aa, Homo sapiens
NWVNVISDLKKIEDLIQSMHIDATLYTESDVHPSCKVTAMKCFLLELQVISLESGDASIHDTVENLIILANNSLSSNGNVTESGCKECEELEEKNIKEFLQSFVHIVQMFINTS

SEQ ID NO: 16 - protein, 224 aa, Homo sapiens
EPKSSDKTHTCPPCPAPEAAGGPSVFLFPPKPKDTLMISRTPEVTCVVVDVSHEDPEVKFNWYVDGVEVHNAKTKPREEQYNSTYRVVSVLTVLHQDWLNGKEYKCKVSNKALGAPIEKTISKAKGQPREPQVYTLPPSRDELTKNQVSLTCLVKGFYPSDIAVEWESNGQPENNYKTTPPVLDSDGSFFLYSKLTVDKSRWQQGNVFSCSVMHEALHNHYTQK

SEQ ID NO: 17 - protein, 77 aa, Homo sapiens
ITCPPPMSVEHADIWVKSYSLYSRERYICNSGFKRKAGTSSLTECVLNKATNVAHWTTPSLKCIRDPALVHQRPAPP

SEQ ID NO: 18 - protein, 217 aa, Homo sapiens
EIVLTQSPATLSLSPGERATLSCRASKGVSTSGYSYLHWYQQKPGQAPRLLIYLASYLESGVPARFSGSGSGTDFTLTISSLEPEDFAVYYCQHSRDLPLTFGGGTKVEIKRTVAAPSVFIFPPSDEQLKSGTASWCLLNNFYPREAKVQWKVDNALQSGNSQESVTEQDSKDSTYSLSSTLTLSKADYEKHKVYACEVTHQGLSSPVTKSFNRGEC

SEQ ID NO: 19 - protein, 214 aa, Homo sapiens
EIVLTQSPATLSLSPGERATLSCRASQSVSSYLAWYQQKPGQAPRLLIYDASNRATGIPARFSGSGSGTDFTLTISSLEPEDFAVYYCQQSSNWPRTFGQGTKVEIKRTVAAPSVFIFPPSDEQLKSGTASVVCLLNNFYPREAKVQWKVDNALQSGNSQESVTEQDSKDSTYSLSSTLTLSKADYEKHKVYACEVTHQGLSSPVTKSFNRGEC

SEQ ID NO: 20 - protein, 217 aa, Homo sapiens
QVQLVQSGVEVKKPGASVKVSCKASGYTFTNYYMYWVRQAPGQGLEWMGGINPSNGGTNFNEKFKNRVTLTTDSSTTTAYMELKSLQFDDTAVYYCARRDYRFDMGFDYWGQGTTVTVSSASTKGPSVFPLAPCSRSTSESTAALGCLVKDYFPEPVTVSWNSGALTSGVHTFPAVLQSSGLYSLSSWTVPSSSLGTKTYTCNVDHKPSNTKVDKRV

SEQ ID NO: 21 - protein, 214 aa, Homo sapiens
QVQLVESGGGVVQPGRSLRLDCKASGITFSNSGMHWVRQAPGKGLEWVAVIWYDGSKRYYADSVKGRFTISRDNSKNTLFLQMNSLRAEDTAVYYCATNDDYWGQGTLVTVSSASTKGPSVFPLAPCSRSTSESTAALGCLVKDYFPEPVTVSWNSGALTSGVHTFPAVLQSSGLYSLSSVVTVPSSSLGTKTYTCNVDHKPSNTKVDKRVESK